European Patent Specification EP 3 077 412 B1, published January 4, 2023. Title: IDENTIFICATION OF A NEW POLYPEPTIDE HORMONE FOR MAINTENANCE OF OPTIMAL BODY WEIGHT AND BLOOD GLUCOSE. Applicant: Chopra, Atul Moore, David. Application UNKNOWN. The sequence listing filed with the application follows.

SEQUENCE LISTING (4 sequences)

SEQ ID NO: 1 - protein, 140 aa, Homo sapiens
STNETDASNIEDQSETEANVSLASWDVEKTAIFAFNISHVSNKVRILELLPALTTLTNHNRYLIESGNEDGFFKINQKEGISYLHFTKKKPVAGTYSLQISSTPLYKKKELNQLEDKYDKDYLSGELGDNLKMKIQVLLH

SEQ ID NO: 2 - protein, 147 aa, Escherichia coli
MHHHHHHSTNETDASNIEDQSETEANVSLASWDVEKTAIFAFNISHVSNKVRILELLPALTTLTNHNRYLIESGNEDGFFKINQKEGISYLHFTKKKPVAGTYSLQISSTPLYKKKELNQLEDKYDKDYLSGELGDNLKMKIQVLLH

SEQ ID NO: 3 - protein, 25 aa, Artificial Sequence
  Synthetic Peptide
ETEANVSLASWDVEKTAIFAFNISH

SEQ ID NO: 4 - protein, 28 aa, Artificial Sequence
  Synthetic Peptide
KKKELNQLEDKYDKDYLSGELGDNLKMK